European Patent Application EP 4 206 219 A1, published July 5, 2023. Title: Fusion Protein Comprising IL15 protein, IL15 receptor alpha protein, Fc domain and IL12 Protein And Uses Thereof. Applicant: GI Cell, Inc. The sequence listing filed with the application follows.

SEQUENCE LISTING (13 sequences)

SEQ ID NO: 1 - protein, 114 aa, Artificial Sequence
  Human IL15
NWVNVISDLKKIEDLIQSMHIDATLYTESDVHPSCKVTAMKCFLLELQVISLESGDASIHDTVENLIILANNSLSSNGNVTESGCKECEELEEKNIKEFLQSFVHIVQMFINTS

SEQ ID NO: 2 - protein, 20 aa, Artificial Sequence
  Linker 1
GGGGSGGGGSGGGGSGGGGS

SEQ ID NO: 3 - protein, 78 aa, Artificial Sequence
  Human IL15Ra  Sushi domain
ITCPPPMSVEHADIWVKSYSLYSRERYICNSGFKRKAGTSSLTECVLNKATNVAHWTTPSLKCIRDPALVHQRPAPPS

SEQ ID NO: 4 - protein, 28 aa, Artificial Sequence
  Linker 2
GGGGSGGGGSGGGGSAESKYGPPCPPCP

SEQ ID NO: 5 - protein, 216 aa, Artificial Sequence
  IgG4 Fc
APEAAGGPSVFLFPPKPKDTLMISRTPEVTCVVVDVSQEDPEVQFNWYVDGVEVHNAKTKPREEQFNSTYRVVSVLTVLHQDWLNGKEYKCKVSNKGLPSSIEKTISKAKGQPREPQVYTLPPSQEEMTKNQVSLTCLVKGFYPSDIAVEWESNGQPENNYKTTPPVLDSDGSFFLYSRLTVDKSRWQEGNVFSCSVMHEALHNHYTQKSLSLSLG

SEQ ID NO: 6 - protein, 5 aa, Artificial Sequence
  Linker 3
GGGGS

SEQ ID NO: 7 - protein, 133 aa, Artificial Sequence [sequence omitted]

SEQ ID NO: 8 - protein, 133 aa, Artificial Sequence
  Human IL2(Mutant)
APTSSSTKKTQLQLEHLLLDLQMILNGINNYKNPKLTAMLTAKFYMPKKATELKHLQCLEEELKPLEEVLNLAQSKNFHLRPRDLISNINVIVLELKGSETTFMCEYADETATIVEFLNRWITFCQSIISTLT

SEQ ID NO: 9 - protein, 594 aa, Artificial Sequence
  Fusion protein A
NWVNVISDLKKIEDLIQSMHIDATLYTESDVHPSCKVTAMKCFLLELQVISLESGDASIHDTVENLIILANNSLSSNGNVTESGCKECEELEEKNIKEFLQSFVHIVQMFINTSGGGGSGGGGSGGGGSGGGGSITCPPPMSVEHADIWVKSYSLYSRERYICNSGFKRKAGTSSLTECVLNKATNVAHWTTPSLKCIRDPALVHQRPAPPSGGGGSGGGGSGGGGSAESKYGPPCPPCPAPEAAGGPSVFLFPPKPKDTLMISRTPEVTCVVVDVSQEDPEVQFNWYVDGVEVHNAKTKPREEQFNSTYRVVSVLTVLHQDWLNGKEYKCKVSNKGLPSSIEKTISKAKGQPREPQVYTLPPSQEEMTKNQVSLTCLVKGFYPSDIAVEWESNGQPENNYKTTPPVLDSDGSFFLYSRLTVDKSRWQEGNVFSCSVMHEALHNHYTQKSLSLSLGGGGGSAPTSSSTKKTQLQLEHLLLDLQMILNGINNYKNPKLTRMLTFKFYMPKKATELKHLQCLEEELKPLEEVLNLAQSKNFHLRPRDLISNINVIVLELKGSETTFMCEYADETATIVEFLNRWITFCQSIISTLT

SEQ ID NO: 10 - protein, 594 aa, Artificial Sequence
  Fusion protein B
NWVNVISDLKKIEDLIQSMHIDATLYTESDVHPSCKVTAMKCFLLELQVISLESGDASIHDTVENLIILANNSLSSNGNVTESGCKECEELEEKNIKEFLQSFVHIVQMFINTSGGGGSGGGGSGGGGSGGGGSITCPPPMSVEHADIWVKSYSLYSRERYICNSGFKRKAGTSSLTECVLNKATNVAHWTTPSLKCIRDPALVHQRPAPPSGGGGSGGGGSGGGGSAESKYGPPCPPCPAPEAAGGPSVFLFPPKPKDTLMISRTPEVTCVVVDVSQEDPEVQFNWYVDGVEVHNAKTKPREEQFNSTYRVVSVLTVLHQDWLNGKEYKCKVSNKGLPSSIEKTISKAKGQPREPQVYTLPPSQEEMTKNQVSLTCLVKGFYPSDIAVEWESNGQPENNYKTTPPVLDSDGSFFLYSRLTVDKSRWQEGNVFSCSVMHEALHNHYTQKSLSLSLGGGGGSAPTSSSTKKTQLQLEHLLLDLQMILNGINNYKNPKLTAMLTAKFYMPKKATELKHLQCLEEELKPLEEVLNLAQSKNFHLRPRDLISNINVIVLELKGSETTFMCEYADETATIVEFLNRWITFCQSIISTLT

SEQ ID NO: 11 - DNA, 1855 bp, Artificial Sequence
  Fusion protein A
gccaccatgaagtgggtcaccttcatctccctgctgtttctgttctcctccgcctactccaactgggtcaacgtgatctccgacctgaagaagatcgaggacctgatccagtccatgcacatcgacgctaccctgtacaccgagtccgatgtgcacccttcttgcaaagtgaccgctatgaagtgcttcctgctggaactgcaagtgatctccctggaatccggcgacgcctctatccacgataccgtggaaaacctgatcatcctggccaacaactccctgtcctccaacggcaatgtgaccgagtctggctgcaaagagtgcgaggaactggaagagaagaacatcaaagagttcctccagtccttcgtccacatcgtgcagatgttcatcaacacctctggcggcggaggaagtggtggcggaggatctggcggtggtggttctggcggaggcggatctattacctgtccacctcctatgtccgtggaacacgccgacatctgggtcaagtcctacagcctgtactccagagagcggtacatctgcaactccggcttcaagagaaaggccggcacatcttctctgaccgagtgcgtgctgaacaaggccaccaatgtggctcactggaccacacctagcctgaagtgcatcagagatcccgctctggtccatcagaggcctgctcctccaagcggtggtggtggaagcggaggtggcggatcaggtggtggcggttctgctgagtctaagtacggacctccttgtccaccttgtcctgctccagaagctgctggcggaccaagcgttttcctgtttcctccaaagcctaaggacaccctgatgatctctcggacccctgaagtgacctgcgtggtggtcgatgtgtctcaagaggaccccgaggtgcagttcaattggtacgtggacggcgtggaagtgcacaacgccaagaccaagcctagagaggaacagttcaactccacctacagagtggtgtccgtgctgaccgtgctgcaccaggattggctgaacggcaaagagtacaagtgcaaggtgtccaacaagggcctgccttccagcatcgaaaagaccatctccaaggctaagggccagcctcgggaacctcaggtttacaccctgcctccaagccaagaggaaatgaccaagaaccaggtgtccctgacctgcctggtcaagggcttctacccttccgatatcgccgtggaatgggagtccaatggccagcctgagaacaactacaagacaacccctcctgtgctggactccgacggctccttttttctgtactcccgcctgaccgtggacaagtccagatggcaagagggcaacgtgttctcctgctctgtgatgcacgaggccctgcacaaccactacacccagaagtccctgtctctgtctcttggaggcggtggcggaagtgctcctacctccagctctaccaagaaaacccagctgcagttggagcatctgctgctggacctccagatgatcctgaatggcatcaacaattacaagaaccccaagctgacccggatgctgaccttcaagttctacatgcccaagaaggccaccgagctgaagcacctccagtgcctggaagaggaactgaagcccctggaagaagtgctgaatctggcccagtccaagaacttccacctgaggcctcgggatctgatctccaacatcaatgtgatcgtgttggagctgaagggctccgagacaaccttcatgtgcgagtacgccgacgagacagccaccatcgtggaatttctgaaccggtggatcaccttctgccagtccatcatctccacactgacctgatgactcgaga

SEQ ID NO: 12 - DNA, 1842 bp, Artificial Sequence
  Fusion protein B
gccaccatgaaatgggtcacctttatctccctgctgttcctgttctcctccgcctactccaactgggtcaacgtgatctccgacctgaagaagatcgaggacctgatccagtccatgcacatcgacgctaccctgtacaccgagtccgacgtgcacccttcctgtaaagtgaccgccatgaagtgctttctgctggaactgcaagtgatctccctggaatccggcgacgcctctatccacgacaccgtggaaaacctgatcatcctggccaacaactccctgtcctccaacggcaacgtgaccgagtctggctgcaaagagtgcgaggaactggaagagaagaacatcaaagagttcctccagtccttcgtgcacatcgtgcagatgttcatcaacacctctggcggcggaggatctggcggaggtggaagcggaggcggaggtagcggtggtggtggatctatcacatgccctccacctatgtccgtggaacacgccgacatctgggtcaagtcctacagcctgtactccagagagcggtacatctgcaactccggcttcaagagaaaggccggcacctctagcctgaccgagtgcgtgctgaacaaggccaccaatgtggcccactggaccacacctagcctgaagtgcatcagggaccccgctctggttcatcagaggcctgctccacctagtggtggcggtggtagtggcggaggcggttcaggtggcggcggatctgctgagtctaagtacggacctccttgtccaccttgtcctgctccagaagctgctggcggcccttccgtgtttctgttccctccaaagcctaaggacaccctgatgatctctcggacccctgaagtgacctgcgtggtggtcgatgtgtcccaagaggatcccgaggtgcagttcaattggtacgtggacggcgtggaagtgcacaacgccaagaccaagcctagagaggaacagttcaactccacctacagagtggtgtccgtgctgaccgtgctgcaccaggattggctgaacggcaaagagtacaagtgcaaggtgtccaacaagggcctgccttccagcatcgaaaagaccatctccaaggccaagggccagcctagggaaccccaggtttacaccctgcctccaagccaagaggaaatgaccaagaaccaggtgtccctgacctgcctggtcaagggcttctacccttccgatatcgccgtggaatgggagagcaatggccagcctgagaacaactacaagacaacccctcctgtgctggactccgacggctccttctttctgtactcccgcctgaccgtggacaagtccagatggcaagagggcaacgtgttctcctgctccgtgatgcacgaggccctgcacaatcactacacccagaagtccctgtctctgtcccttggaggtggtggtggctctgctcctacctcctccagcaccaagaaaacccagctgcagttggagcatctgctgctggacctccagatgatcctgaatggcatcaacaattacaagaaccccaagctcaccgccatgctgaccgccaagttctacatgcccaagaaggccaccgagctgaagcacctccagtgcctggaagaggaactgaagcccctggaagaagtgctgaatctggcccagtccaagaacttccacctgaggcctcgcgacctgatctccaacatcaatgtgatcgtgttggagctgaagggctccgagacaaccttcatgtgcgagtacgccgacgagacagctaccatcgtggaatttctgaaccggtggatcaccttctgccagtccatcatctccacactgacc

SEQ ID NO: 13 - protein, 18 aa, Artificial Sequence
  Albumin Signal Sequence
MKWVTFISLLFLFSSAYS